European Patent Application EP 4 219 727 A2, published August 2, 2023. Title: PRODUCTS AND METHODS FOR TREATMENT OF AMYOTROPHIC LATERAL SCLEROSIS. Applicant: Research Institute at Nationwide Children's Hospital. The sequence listing filed with the application follows.

SEQUENCE LISTING (22 sequences)

SEQ ID NO: 1 - DNA, 26 bp, synthetic construct
  source 1..26: mol_type = other DNA
gcatcatcaatttcgagcagaaggaa

SEQ ID NO: 2 - DNA, 23 bp, synthetic construct
  source 1..23: mol_type = other DNA
gaagcattaaaggactgactgaa

SEQ ID NO: 3 - DNA, 23 bp, synthetic construct
  source 1..23: mol_type = other DNA
ctgactgaaggcctgcatggatt

SEQ ID NO: 4 - DNA, 20 bp, synthetic construct
  source 1..20: mol_type = other DNA
catggattccatgttcatga

SEQ ID NO: 5 - DNA, 21 bp, synthetic construct
  source 1..21: mol_type = other DNA
gcatggattccatgttcatga

SEQ ID NO: 6 - DNA, 21 bp, synthetic construct
  source 1..21: mol_type = other DNA
ggtctggcctataaagtagtc

SEQ ID NO: 7 - DNA, 21 bp, synthetic construct
  source 1..21: mol_type = other DNA
gggcatcatcaatttcgagca

SEQ ID NO: 8 - DNA, 21 bp, synthetic construct
  source 1..21: mol_type = other DNA
gcatcatcaatttcgagcaga

SEQ ID NO: 9 - DNA, 21 bp, synthetic construct
  source 1..21: mol_type = other DNA
gcctgcatggattccatgttc

SEQ ID NO: 10 - DNA, 21 bp, synthetic construct
  source 1..21: mol_type = other DNA
ggaggtctggcctataaagta

SEQ ID NO: 11 - DNA, 21 bp, synthetic construct
  source 1..21: mol_type = other DNA
gattccatgttcatgagtttg

SEQ ID NO: 12 - DNA, 21 bp, synthetic construct
  source 1..21: mol_type = other DNA
ggagataatacagcaggctgt

SEQ ID NO: 13 - DNA, 21 bp, synthetic construct
  source 1..21: mol_type = other DNA
gctttaaagtacctgtagtga

SEQ ID NO: 14 - DNA, 21 bp, synthetic construct
  source 1..21: mol_type = other DNA
gcattaaaggactgactgaag

SEQ ID NO: 15 - DNA, 19 bp, synthetic construct
  source 1..19: mol_type = other DNA
tcatcaatttcgagcagaa

SEQ ID NO: 16 - DNA, 19 bp, synthetic construct
  source 1..19: mol_type = other DNA
tcgagcagaaggaaagtaa

SEQ ID NO: 17 - DNA, 19 bp, synthetic construct
  source 1..19: mol_type = other DNA
gcctgcatggattccatgt

SEQ ID NO: 18 - DNA, 19 bp, synthetic construct
  source 1..19: mol_type = other DNA
tcactctcaggagaccatt

SEQ ID NO: 19 - DNA, 19 bp, synthetic construct
  source 1..19: mol_type = other DNA
gctttaaagtacctgtagt

SEQ ID NO: 20 - DNA, 5786 bp, synthetic construct
  source 1..5786: mol_type = other DNA
gcccaatacgcaaaccgcctctccccgcgcgttggccgattcattaatgcagctgattctaacgaggaaagcacgttatacgtgctcgtcaaagcaaccatagtacgcgccctgtagcggcgcattaagcgcggcgggtgtggtggttacgcgcagcgtgaccgctacacttgccagcgccctagcgcccgctcctttcgctttcttcccttcctttctcgccacgttcgccggctttccccgtcaagctctaaatcgggggctccctttagggttccgatttagtgctttacggcacctcgaccccaaaaaacttgattagggtgatggttcacgtagtgggccatcgccctgatagacggtttttcgccctttgacgttggagtccacgttctttaatagtggactcttgttccaaactggaacaacactcaaccctatctcggtctattcttttgatttataagggattttgccgatttcggcctattggttaaaaaatgagctgatttaacaaaaatttaacgcgaattttaacaaaatattaacgcttacaatttaaatatttgcttatacaatcttcctgtttttggggcttttctgattatcaaccggggtacatatgattgacatgctagttttacgattaccgttcatcgccctgcgcgctcgctcgctcactgaggccgcccgggcaaagcccgggcgtcgggcgacctttggtcgcccggcctcagtgagcgagcgagcgcgcagagagggagtggaattcacgcgtggatctgaattcaattcacgcgtggtacctacactttatgcttccggctcgtatgttgtgtggaattgtgagcggataacaatttcacacaggaaacagctatgaccatgattacgccaagctttccaaaaaagcatggattccatgttcatgatctcttgaatcatgaacatggaatccatggatccgagtggtctcatacagaacttataagattcccaaatccaaagacatttcacgtttatggtgatttcccagaacacatagcgacatgcaaatatgaattcactggccgtcgttttacaacgtcgtgactgggaaaaccctggcgttacccaacttaatcgccttgcagcacatccccctttcgccagctggcgtaatagcgaagaggcccgcaccgatcgcccttcccaacagttgcgcagcctgtggtacctctggtcgttacataacttacggtaaatggcccgcctggctgaccgcccaacgacccccgcccattgacgtcaataatgacgtatgttcccatagtaacgccaatagggactttccattgacgtcaatgggtggagtatttacggtaaactgcccacttggcagtacatcaagtgtatcatatgccaagtacgccccctattgacgtcaatgacggtaaatggcccgcctggcattatgcccagtacatgaccttatgggactttcctacttggcagtacatctactcgaggccacgttctgcttcactctccccatctcccccccctccccacccccaattttgtatttatttattttttaattattttgtgcagcgatgggggcggggggggggggggggcgcgcgccaggcggggcggggcggggcgaggggcggggcggggcgaggcggagaggtgcggcggcagccaatcagagcggcgcgctccgaaagtttccttttatggcgaggcggcggcggcggcggccctataaaaagcgaagcgcgcggcgggcgggagcgggatcagccaccgcggtggcggcctagagtcgacgaggaactgaaaaaccagaaagttaactggtaagtttagtctttttgtcttttatttcaggtcccggatccggtggtggtgcaaatcaaagaactgctcctcagtggatgttgcctttacttctaggcctgtacggaagtgttacttctgctctaaaagctgcggaattgtacccgcggccgatccaccggtcgccaccatggtgagcaagggcgaggagctgttcaccggggtggtgcccatcctggtcgagctggacggcgacgtaaacggccacaagttcagcgtgtccggcgagggcgagggcgatgccacctacggcaagctgaccctgaagttcatctgcaccaccggcaagctgcccgtgccctggcccaccctcgtgaccaccctgacctacggcgtgcagtgcttcagccgctaccccgaccacatgaagcagcacgacttcttcaagtccgccatgcccgaaggctacgtccaggagcgcaccatcttcttcaaggacgacggcaactacaagacccgcgccgaggtgaagttcgagggcgacaccctggtgaaccgcatcgagctgaagggcatcgacttcaaggaggacggcaacatcctggggcacaagctggagtacaactacaacagccacaacgtctatatcatggccgacaagcagaagaacggcatcaaggtgaacttcaagatccgccacaacatcgaggacggcagcgtgcagctcgccgaccactaccagcagaacacccccatcggcgacggccccgtgctgctgcccgacaaccactacctgagcacccagtccgccctgagcaaagaccccaacgagaagcgcgatcacatggtcctgctggagttcgtgaccgccgccgggatcactctcggcatggacgagctgtacaagtaaagcggccatcaagcttatcgataccgtcgactagagctcgctgatcagcctcgactgtgccttctagttgccagccatctgttgtttgcccctcccccgtgccttccttgaccctggaaggtgccactcccactgtcctttcctaataaaatgaggaaattgcatcgcattgtctgagtaggtgtcattctattctggggggtggggtggggcaggacagcaagggggaggattgggaagacaatagcaggcatgctggggagagatcgatctgaggaacccctagtgatggagttggccactccctctctgcgcgctcgctcgctcactgaggccgggcgaccaaaggtcgcccgacgcccgggctttgcccgggcggcctcagtgagcgagcgagcgcgcagagagggagtggcccccccccccccccccccggcgattctcttgtttgctccagactctcaggcaatgacctgatagcctttgtagagacctctcaaaaatagctaccctctccggcatgaatttatcagctagaacggttgaatatcatattgatggtgatttgactgtctccggcctttctcacccgtttgaatctttacctacacattactcaggcattgcatttaaaatatatgagggttctaaaaatttttatccttgcgttgaaataaaggcttctcccgcaaaagtattacagggtcataatgtttttggtacaaccgatttagctttatgctctgaggctttattgcttaattttgctaattctttgccttgcctgtatgatttattggatgttggaatcgcctgatgcggtattttctccttacgcatctgtgcggtatttcacaccgcatatggtgcactctcagtacaatctgctctgatgccgcatagttaagccagccccgacacccgccaacacccgctgacgcgccctgacgggcttgtctgctcccggcatccgcttacagacaagctgtgaccgtctccgggagctgcatgtgtcagaggttttcaccgtcatcaccgaaacgcgcgagacgaaagggcctcgtgatacgcctatttttataggttaatgtcatgataataatggtttcttagacgtcaggtggcacttttcggggaaatgtgcgcggaacccctatttgtttatttttctaaatacattcaaatatgtatccgctcatgagacaataaccctgataaatgcttcaataatattgaaaaaggaagagtatgagtattcaacatttccgtgtcgcccttattcccttttttgcggcattttgccttcctgtttttgctcacccagaaacgctggtgaaagtaaaagatgctgaagatcagttgggtgcacgagtgggttacatcgaactggatctcaacagcggtaagatccttgagagttttcgccccgaagaacgttttccaatgatgagcacttttaaagttctgctatgtggcgcggtattatcccgtattgacgccgggcaagagcaactcggtcgccgcatacactattctcagaatgacttggttgagtactcaccagtcacagaaaagcatcttacggatggcatgacagtaagagaattatgcagtgctgccataaccatgagtgataacactgcggccaacttacttctgacaacgatcggaggaccgaaggagctaaccgcttttttgcacaacatgggggatcatgtaactcgccttgatcgttgggaaccggagctgaatgaagccataccaaacgacgagcgtgacaccacgatgcctgtagcaatggcaacaacgttgcgcaaactattaactggcgaactacttactctagcttcccggcaacaattaatagactggatggaggcggataaagttgcaggaccacttctgcgctcggcccttccggctggctggtttattgctgataaatctggagccggtgagcgtgggtctcgcggtatcattgcagcactggggccagatggtaagccctcccgtatcgtagttatctacacgacggggagtcaggcaactatggatgaacgaaatagacagatcgctgagataggtgcctcactgattaagcattggtaactgtcagaccaagtttactcatatatactttagattgatttaaaacttcatttttaatttaaaaggatctaggtgaagatcctttttgataatctcatgaccaaaatcccttaacgtgagttttcgttccactgagcgtcagaccccgtagaaaagatcaaaggatcttcttgagatcctttttttctgcgcgtaatctgctgcttgcaaacaaaaaaaccaccgctaccagcggtggtttgtttgccggatcaagagctaccaactctttttccgaaggtaactggcttcagcagagcgcagataccaaatactgtccttctagtgtagccgtagttaggccaccacttcaagaactctgtagcaccgcctacatacctcgctctgctaatcctgttaccagtggctgctgccagtggcgataagtcgtgtcttaccgggttggactcaagacgatagttaccggataaggcgcagcggtcgggctgaacggggggttcgtgcacacagcccagcttggagcgaacgacctacaccgaactgagatacctacagcgtgagctatgagaaagcgccacgcttcccgaagggagaaaggcggacaggtatccggtaagcggcagggtcggaacaggagagcgcacgagggagcttccagggggaaacgcctggtatctttatagtcctgtcgggtttcgccacctctgacttgagcgtcgatttttgtgatgctcgtcaggggggcggagcctatggaaaaacgccagcaacgcggcctttttacggttcctggccttttgctggccttttgctcacatgttctttcctgcgttatcccctgattctgtggataaccgtattaccgcctttgagtgagctgataccgctcgccgcagccgaacgaccgagcgcagcgagtcagtgagcgaggaagcggaagagc

SEQ ID NO: 21 - DNA, 164 bp, synthetic construct
  source 1..164: mol_type = other DNA
aattcatatttgcatgtcgctatgtgttctgggaaatcaccataaacgtgaaatgtctttggatttgggaatcttataagttctgtatgagaccactcggatccatggattccatgttcatgattcaagagatcatgaacatggaatccatgcttttttggaaa

SEQ ID NO: 22 - DNA, 1607 bp, synthetic construct
  source 1..1607: mol_type = other DNA
tctagaggctcgagaagatatcaactgcagcttctactgggcggttttatggacagcaagcgaaccggaattgccagctggggcgccctctggtaaggttgggaagccctgcaaagtaaactggatggctttctcgccgccaaggatctgatggcgcaggggatcaagctctgatcaagagacaggatgaggatcgtttcgcgttcttgactcttcgcgatgtacgggccagatatacgcgttgacattgattattgactagttattaatagtaatcaattacggggtcattagttcatagcccatatatggagttccgcctgcagggacgtcgacggatcgggagatctcccgatcccctatctgctccctgcttgtgtgttggaggtcgctgagtagtgcgcgagcaaaatttaagctacaacaaggcaaggcttgaccgacaattgcatgaagaatctgcttagggttaggcgttttgcgctgcttcgcggcgcgccttttaaggcagttattggtgcccttaaacgcctggtgctacgcctgaataagtgataataagcggatgaatggcagaaattcgccggatctttgtgaaggaaccttacttctgtggtgtgacataattggacaaactacctacagagatttaaagctctaatgtaagcagacagttttattgttcatgatgatatatttttatcttgtgcaatgtaacatcagagattttgagacacaacgtggctttccccccccccccctagggtgggcgaagaactccagcatgagatccccgcgctggaggatcatccagccggcgtcccggaaaacgattccgaagcccaacctttcatagaaggcggcggtggaatcgaaatctcgtgatggcaggttgggcgtcgcttggtcggtcatttcgaaccccagagtcccgctcagggcgcgccgggggggggggcgctgaggtctgcctcgtgaagaaggtgttgctgactcataccaggcctgaatcgccccatcatccagccagaaagtgagggagccacggttgatgagagctttgttgtaggtggaccagtcctgcaggagcataaagtgtaaagcctggggtgcctaatgagtgagctaactcacattaattgcgttgcgctcactgcccgctttccagtcgggaaacctgtcgtgcccgcccagtctagctatcgccatgtaagcccactgcaagctacctgctttctctttgcgcttgcgttttcccttgtccagatagcccagtagctgacattcatccggggtcagcaccgtttctgcggactggctttctacgtgtctggttcgaggcgggatcagccaccgcggtggcggcctagagtcgacgaggaactgaaaaaccagaaagttaactggcctgtacggaagtgttacttctgctctaaaagctgcggaattgtacccgcggccgatccaccggtcgccaccagcggccatcaagcacgttatcgataccgtcgactagagctcgctgatcagtggggggtggggtggggcaggacagcaagggggaggattgggaagacaatagcagctgcagaagtttaaacgcatgc